European Patent Specification EP 3 795 699 B1, published December 20, 2023. Title: DIGITAL SEQUENCE ANALYSIS OF DNA METHYLATION. Applicant: EXACT SCIENCES DEVELOPMENT COMPANY, LLC MAYO FOUNDATION FOR MEDICAL EDUCATION AND RESEARCH. Application EP. The sequence listing filed with the application follows.

SEQUENCE LISTING (15 sequences)

SEQ ID NO: 1 - DNA, 121 bp, Homo sapiens
gaagagcccacctgtcaggctgcgctgggtcagcgcagcaagtggggctggccgctatctcgctgcacccggccgcgtcccgggctccgtgcgccctcgccccagctggtttggagttcaa

SEQ ID NO: 2 - DNA, 121 bp, Artificial
  Synthetic
gaagagtttatttgttaggttgtgttgggttagtgtagtaagtggggttggttgttattttgttgtatttggttgtgttttgggttttgtgtgtttttgttttagttggtttggagtttaa

SEQ ID NO: 3 - DNA, 121 bp, Artificial
  Synthetic
gaagagtttatttgttaggttgcgttgggttagcgtagtaagtggggttggtcgttatttcgttgtattcggtcgcgtttcgggtttcgtgcgttttcgttttagttggtttggagtttaa

SEQ ID NO: 4 - DNA, 129 bp, Homo sapiens
aaataaaaacggagtgggtcccccgcgcgccgccgccccccgcgtccctggcggcctcccccgaggcccccggcggcctcacgagcccgcagtagccggtggcgacgtcgcccccgccccacctccccg

SEQ ID NO: 5 - DNA, 132 bp, Artificial
  Synthetic
gttaaataaaaatggagtgggttttttgtgtgttgttgttttttgtgtttttggtggttttttttgaggtttttggtggttttatgagtttgtagtagttggtggtgatgttgtttttgttttatttttttg

SEQ ID NO: 6 - DNA, 132 bp, Artificial
  Synthetic
gttaaataaaaacggagtgggtttttcgcgcgtcgtcgtttttcgcgtttttggcggtttttttcgaggttttcggcggttttacgagttcgtagtagtcggtggcgacgtcgttttcgttttatttttttg

SEQ ID NO: 7 - DNA, 99 bp, Homo sapiens
ggccgcagcagccagcccagcacccaccttcgaagtccgaaatgatcccatccagctgcgcgttgaccgcggggtccgacatgatggctggtgggcagc

SEQ ID NO: 8 - DNA, 99 bp, Artificial
  Synthetic
ggttgtagtagttagtttagtatttatttttgaagtttgaaatgattttatttagttgtgtgttgattgtggggtttgatatgatggttggtgggtagt

SEQ ID NO: 9 - DNA, 99 bp, Artificial
  Synthetic
ggtcgtagtagttagtttagtatttattttcgaagttcgaaatgattttatttagttgcgcgttgatcgcggggttcgatatgatggttggtgggtagc

SEQ ID NO: 10 - DNA, 116 bp, Homo sapiens
aggaggtgcgcggctttctgctccaggcggcccgggtgcccgctttatgcggggcgagcgtccggccgacccccgccggggcggagcctgaggggtggctgattcatgcacgggga

SEQ ID NO: 11 - DNA, 116 bp, Artificial
  Synthetic
aggaggtgtgtggttttttgttttaggtggtttgggtgtttgttttatgtggggtgagtgtttggttgatttttgttggggtggagtttgaggggtggttgatttatgtatgggga

SEQ ID NO: 12 - DNA, 116 bp, Artificial
  Synthetic
aggaggtgcgcggttttttgttttaggcggttcgggtgttcgttttatgcggggcgagcgttcggtcgattttcgtcggggcggagtttgaggggtggttgatttatgtacgggga

SEQ ID NO: 13 - DNA, 117 bp, Homo sapiens
caggtccgtgtcctcgtcctcctaccgcaggatgttcggcggcccgggcaccgcgagccggccgagctccagccggagctacgtgactacgtccacccgcacctacagcctgggcga

SEQ ID NO: 14 - DNA, 117 bp, Artificial
  Synthetic
taggtttgtgtttttgtttttttattgtaggatgtttggtggtttgggtattgtgagttggttgagttttagttggagttatgtgattatgtttatttgtatttatagtttgggtag

SEQ ID NO: 15 - DNA, 117 bp, Artificial
  Synthetic
taggttcgtgttttcgtttttttatcgtaggatgttcggcggttcgggtatcgcgagtcggtcgagttttagtcggagttacgtgattacgtttattcgtatttatagtttgggtag